European Patent Specification EP 3 843 748 B1, published June 25, 2025. Title: Combination Therapy. Applicant: ADC THERAPEUTICS SA MEDIMMUNE LIMITED. The sequence listing filed with the application follows.

SEQUENCE LISTING (15 sequences)

SEQ ID NO: 1 - protein, 119 aa, Artificial Sequence
  anti-CD19-ADC antibody RB4v1.0 VH
QVQLVQPGAEVVKPGASVKLSCKTSGYTFTSNWMHWVKQRPGQGLEWIGEIDPSDSYTNYNQNFKGKAKLTVDKSTSTAYMEVSSLRSDDTAVYYCARGSNPYYYAMDYWGQGTSVTVS

SEQ ID NO: 2 - protein, 119 aa, Artificial Sequence
  anti-CD19-ADC antibody RB4v1.2 VH
QVQLVQPGAEVVKPGASVKLSCKTSGYTFTSNWMHWVKQAPGQGLEWIGEIDPSDSYTNYNQNFQGKAKLTVDKSTSTAYMEVSSLRSDDTAVYYCARGSNPYYYAMDYWGQGTSVTVS

SEQ ID NO: 3 - protein, 121 aa, Artificial Sequence
  anti-CD19-ADC antibody B43 VH
QVQLLESGAELVRPGSSVKISCKASGYAFSSYWMNWVKQRPGQGLEWIGQIWPGDGDTNYNGKFKGKATLTADESSSTAYMQLSSLRSEDSAVYSCARRETTTVGRYYYAMDYWGQGTTVT

SEQ ID NO: 4 - protein, 123 aa, Artificial Sequence
  anti-CD19-ADC antibody HD37 VH
QVQLQQSGAELVRPGSSVKISCKASGYAFSSYWMNWVKQRPGQGLEWIGQIWPGDGDTNYNGKFKGKATLTADESSSTAYMQLSSLASEDSAVYFCARRETTTVGRYYYAMDYWGQGTSVTVS

SEQ ID NO: 5 - protein, 120 aa, Artificial Sequence
  anti-CD19-ADC antibody 4G7 VH
EVQLQQSGPELIKPGASVKMSCKASGYTFTSYVMHWVKQKPGQGLEWIGYINPYNDGTKYNEKFKGKATLTSDKSSSTAYMELSSLTSEDSAVYYCARGTYYYGSRVFDYWGQGTTLTVS

SEQ ID NO: 6 - protein, 119 aa, Artificial Sequence
  anti-CD19-ADC antibody FMC63 VH
EVKLQESGPGLVAPSQSLSVTCTVSGVSLPDYGVSWIRQPPRKGLEWLGVIWGSETTYYNSALKSRLTIIKDNSKSQVFLKMNSLQTDDTAIYYCAKHYYYGGSYAMDYWGQGTSVTVS

SEQ ID NO: 7 - protein, 104 aa, Artificial Sequence
  anti-CD19-ADC antibody RB4v1.0 VK
EIVLTQSPAIMSASPGERVTMTCSASSGVNYMHWYQQKPGTSPRRWIYDTSKLASGVPARFSGSGSGTSYSLTISSMEPEDAATYYCHQRGSYTFGGGTKLEIK

SEQ ID NO: 8 - protein, 104 aa, Artificial Sequence; identical to SEQ ID NO: 7
  anti-CD19-ADC antibody RB4v1.2 VK

SEQ ID NO: 9 - protein, 111 aa, Artificial Sequence
  anti-CD19-ADC antibody B43 VK
ELVLTQSPASLAVSLGQRATISCKASQSVDYDGDSYLNWYQQIPGQPPKLLIYDASNLVSGIPPRFSGSGSGTDFTLNIHPVEKVDAATYHCQQSTEDPWTFGGGTKLEIK

SEQ ID NO: 10 - protein, 111 aa, Artificial Sequence
  anti-CD19-ADC antibody HD37 VK
DILLTQTPASLAVSLGQRATISCKASQSVDYDGDSYLNWYQQIPGQPPKLLIYDASNLVSGIPPRFSGSGSGTDFTLNIHPVEKVDAATYHCQQSTEDPWTFGGGTKLEIK

SEQ ID NO: 11 - protein, 112 aa, Artificial Sequence
  anti-CD19-ADC antibody 4G7 VK
DIVMTQAAPSIPVTPGESVSISCRSSKSLLNSNGNTYLYWFLQRPGQSPQLLIYRMSNLASGVPDRFSGSGSGTAFTLRISRVEAEDVGVYYCMQHLEYPFTFGAGTKLELK

SEQ ID NO: 12 - protein, 107 aa, Artificial Sequence
  anti-CD19-ADC antibody FMC63 VK
DIQMTQTTSSLSASLGDRVTISCRASQDISKYLNWYQQKPDGTVKLLIYHTSRLHSGVPSRFSGSGSGTDYSLTISNLEQEDIATYFCQQGNTLPYTFGGGTKLEIT

SEQ ID NO: 13 - protein, 449 aa, Artificial Sequence
  anti-CD19-ADC antibody RB4v1.2-HC
QVQLVQPGAEVVKPGASVKLSCKTSGYTFTSNWMHWVKQAPGQGLEWIGEIDPSDSYTNYNQNFQGKAKLTVDKSTSTAYMEVSSLRSDDTAVYYCARGSNPYYYAMDYWGQGTSVTVSSASTKGPSVFPLAPSSKSTSGGTAALGCLVKDYFPEPVTVSWNSGALTSGVHTFPAVLQSSGLYSLSSVVTVPSSSLGTQTYICNVNHKPSNTKVDKKVEPKSCDKTHTCPPCPAPELLGGPSVFLFPPKPKDTLMISRTPEVTCVVVDVSHEDPEVKFNWYVDGVEVHNAKTKPREEQYNSTYRVVSVLTVLHQDWLNGKEYKCKVSNKALPAPIEKTISKAKGQPREPQVYTLPPSREEMTKNQVSLTCLVKGFYPSDIAVEWESNGQPENNYKTTPPVLDSDGSFFLYSKLTVDKSRWQQGNVFSCSVMHEALHNHYTQKSLSLSPG

SEQ ID NO: 14 - protein, 211 aa, Artificial Sequence
  anti-CD19-ADC antibody RB4v1.2-LC
EIVLTQSPAIMSASPGERVTMTCSASSGVNYMHWYQQKPGTSPRRWIYDTSKLASGVPARFSGSGSGTSYSLTISSMEPEDAATYYCHQRGSYTFGGGTKLEIKRTVAAPSVFIFPPSDEQLKSGTASVVCLLNNFYPREAKVQWKVDNALQSGNSQESVTEQDSKDSTYSLSSTLTLSKADYEKHKVYACEVTHQGLSSPVTKSFNRGEC

SEQ ID NO: 15 - DNA, 18 bp, Artificial Sequence
  oblimersen (G3139) oligo structure
tctcccagcgtgcgccat